European Patent Application EP 4 435 101 A1, published September 25, 2024. Title: MEMBRANE SURFACE PROTEIN CONTAINING GPI ANCHOR REGION. Applicant: Shanghai Juncell Therapeutics Co., Ltd. Application EP 22894779.2, filed November 15, 2022. The sequence listing filed with the application follows.

SEQUENCE LISTING (20 sequences)

SEQ ID NO: 1 - DNA, 807 bp, synthetic construct
  misc_feature 1..807: note = encoding nucleic acids
  source 1..807: mol_type = other DNA
atgaagcgcttcctcttcctcctactcaccatcagcctcctggttatggtacagatacaaactggactctcagattgtgatattgaaggtaaagatggcaaacaatatgagagtgttctaatggtcagcatcgatcaattattggacagcatgaaagaaattggtagcaattgcctgaataatgaatttaacttttttaaaagacatatctgtgatgctaataaggaaggtatgtttttattccgtgctgctcgcaagttgaggcaatttcttaaaatgaatagcactggtgattttgatctccacttattaaaagtttcagaaggcacaacaatactgttgaactgcactggccaggttaaaggaagaaaaccagctgccctgggtgaagcccaaccaacaaagagtttggaagaaaataaatctttaaaggaacagaaaaaactgaatgacttgtgtttcctaaagagactattacaagagataaaaacttgttggaataaaattttgatgggcactaaagaacacttcgtgccggtcttcctgccagcgaagcccaccacgacgccagcgccgcgaccaccaacaccggcgcccaccatcgcgtcgcagcccctgtccctgcgcccagaggcgtgccggccagcggcggggggcgcagtgcacacgagggggctggacttcgcctgtgatggacaaaacgacaccagccaaaccagcagcccctcagcatccagcaacataagcggaggcattttccttttcttcgtggccaatgccataatccacctcttctgcttcagttga

SEQ ID NO: 2 - protein, 268 aa, synthetic construct
  REGION 1..268: note = fusion protein
MKRFLFLLLTISLLVMVQIQTGLSDCDIEGKDGKQYESVLMVSIDQLLDSMKEIGSNCLNNEFNFFKRHICDANKEGMFLFRAARKLRQFLKMNSTGDFDLHLLKVSEGTTILLNCTGQVKGRKPAALGEAQPTKSLEENKSLKEQKKLNDLCFLKRLLQEIKTCWNKILMGTKEHFVPVFLPAKPTTTPAPRPPTPAPTIASQPLSLRPEACRPAAGGAVHTRGLDFACDGQNDTSQTSSPSASSNISGGIFLFFVANAIIHLFCFS

SEQ ID NO: 3 - DNA, 840 bp, synthetic construct
  misc_feature 1..840: note = encoding nucleic acids
  source 1..840: mol_type = other DNA
atgaagcgcttcctcttcctcctactcaccatcagcctcctggttatggtacagatacaaactggactctcagattgtgatattgaaggtaaagatggcaaacaatatgagagtgttctaatggtcagcatcgatcaattattggacagcatgaaagaaattggtagcaattgcctgaataatgaatttaacttttttaaaagacatatctgtgatgctaataaggaaggtatgtttttattccgtgctgctcgcaagttgaggcaatttcttaaaatgaatagcactggtgattttgatctccacttattaaaagtttcagaaggcacaacaatactgttgaactgcactggccaggttaaaggaagaaaaccagctgccctgggtgaagcccaaccaacaaagagtttggaagaaaataaatctttaaaggaacagaaaaaactgaatgacttgtgtttcctaaagagactattacaagagataaaaacttgttggaataaaattttgatgggcactaaagaacacgccgaggccgccgccaaggaggccgccgccaaggccatgttgcagatggctgggcagtgctcccaaaatgaatattttgacagtttgttgcatgcttgcataccttgtcaacttcgatgttcttctaatactcctcctctaacatgtcagcgttattgtaatgcaagtgtgaccaattcagtgaaaggaacgaatgcgggacaaaacgacaccagccaaaccagcagcccctcagcatccagcaacataagcggaggcattttccttttcttcgtggccaatgccataatccacctcttctgcttcagttga

SEQ ID NO: 4 - protein, 279 aa, synthetic construct
  REGION 1..279: note = fusion protein
MKRFLFLLLTISLLVMVQIQTGLSDCDIEGKDGKQYESVLMVSIDQLLDSMKEIGSNCLNNEFNFFKRHICDANKEGMFLFRAARKLRQFLKMNSTGDFDLHLLKVSEGTTILLNCTGQVKGRKPAALGEAQPTKSLEENKSLKEQKKLNDLCFLKRLLQEIKTCWNKILMGTKEHAEAAAKEAAAKAMLQMAGQCSQNEYFDSLLHACIPCQLRCSSNTPPLTCQRYCNASVTNSVKGTNAGQNDTSQTSSPSASSNISGGIFLFFVANAIIHLFCFS

SEQ ID NO: 5 - DNA, 759 bp, synthetic construct
  misc_feature 1..759: note = encoding nucleic acids
  source 1..759: mol_type = other DNA
atggccttaccagtgaccgccttgctcctgccgctggccttgctgctccacgccgccaggccggattgtgatattgaaggtaaagatggcaaacaatatgagagtgttctaatggtcagcatcgatcaattattggacagcatgaaagaaattggtagcaattgcctgaataatgaatttaacttttttaaaagacatatctgtgatgctaataaggaaggtatgtttttattccgtgctgctcgcaagttgaggcaatttcttaaaatgaatagcactggtgattttgatctccacttattaaaagtttcagaaggcacaacaatactgttgaactgcactggccaggttaaaggaagaaaaccagctgccctgggtgaagcccaaccaacaaagagtttggaagaaaataaatctttaaaggaacagaaaaaactgaatgacttgtgtttcctaaagagactattacaagagataaaaacttgttggaataaaattttgatgggcactaaagaacacttcgtgccggtcttcctgccagcgaagcccaccacgacgccagcgccgcgaccaccaacaccggcgcccaccatcgcgtcgcagcccctgtccctgcgcccagaggcgtgccggccagcggcggggggcgcagtgcacacgagggggctggacttcgcctgtgatatctacatctgggcgcccctggccgggacttgtggggtccttctcctgtcactggttatcaccctttactgctga

SEQ ID NO: 6 - protein, 252 aa, synthetic construct
  REGION 1..252: note = fusion protein
MALPVTALLLPLALLLHAARPDCDIEGKDGKQYESVLMVSIDQLLDSMKEIGSNCLNNEFNFFKRHICDANKEGMFLFRAARKLRQFLKMNSTGDFDLHLLKVSEGTTILLNCTGQVKGRKPAALGEAQPTKSLEENKSLKEQKKLNDLCFLKRLLQEIKTCWNKILMGTKEHFVPVFLPAKPTTTPAPRPPTPAPTIASQPLSLRPEACRPAAGGAVHTRGLDFACDIYIWAPLAGTCGVLLLSLVITLYC

SEQ ID NO: 7 - DNA, 954 bp, synthetic construct
  misc_feature 1..954: note = encoding nucleic acids
  source 1..954: mol_type = other DNA
atgaagcgcttcctcttcctcctactcaccatcagcctcctggttatggtacagatacaaactggactctcagacatccagatgacccagtccccttcctccctctctgcctctgtgggagaccgcgttaccatcacatgccgagcttcccaggacgtgaacacagccgtggcctggtaccagcagaagcccgggaaggcacccaaactcctcatctactccgcctccttcctagagagtggcgtgccttcccgattctccggctccaggagtggcacggactttacgctcaccattagtagcctgcagcccgaagacttcgcgacctactattgtcagcaacactacacgacgccaccaactttcggccagggtaccaaggtcgagattaagcgaaccggcagtaccagtgggtctggcaagcccggcagcggcgagggatccgaggtccagctggtcgagtccggcgggggcctggtgcagccgggcggctcgctgaggttatcttgcgccgccagtggcttcaacatcaaggatacttacatccactgggtgaggcaggctccgggcaagggcctggaatgggtggctaggatctaccctactaacgggtacacacgctacgcagattcggtgaaaggccgcttcactatctccgccgacacctcgaagaacactgcttacctgcagatgaactccctcagggccgaagatactgcagtctactactgctcccgctggggtggggacggcttcgtagccatggacgtgtggggtcagggcactctagttacagtgtcatccgccgaggccgccgccaaggaggccgccgccaaggccggacaaaacgacaccagccaaaccagcagcccctcagcatccagcaacataagcggaggcattttccttttcttcgtggccaatgccataatccacctcttctgcttcagttga

SEQ ID NO: 8 - protein, 317 aa, synthetic construct
  REGION 1..317: note = fusion protein
MKRFLFLLLTISLLVMVQIQTGLSDIQMTQSPSSLSASVGDRVTITCRASQDVNTAVAWYQQKPGKAPKLLIYSASFLESGVPSRFSGSRSGTDFTLTISSLQPEDFATYYCQQHYTTPPTFGQGTKVEIKRTGSTSGSGKPGSGEGSEVQLVESGGGLVQPGGSLRLSCAASGFNIKDTYIHWVRQAPGKGLEWVARIYPTNGYTRYADSVKGRFTISADTSKNTAYLQMNSLRAEDTAVYYCSRWGGDGFVAMDVWGQGTLVTVSSAEAAAKEAAAKAGQNDTSQTSSPSASSNISGGIFLFFVANAIIHLFCFS

SEQ ID NO: 9 - DNA, 957 bp, synthetic construct
  misc_feature 1..957: note = encoding nucleic acids
  source 1..957: mol_type = other DNA
atgaagcgcttcctcttcctcctactcaccatcagcctcctggttatggtacagatacaaactggactctcacaggtgcaactacagcagtggggcgcaggactgttgaagccttcggagaccctgtccctcacctgcgctgtctatggtgggtccttcagtggttactactggagctggatacgccagtccccagagaaggggctggagtggattggggaaatcaatcatggtggatacgtcacctacaatccgtccctcgagagtcgagtcaccatatcagtagacacgtccaagaaccagttctccctgaagctgagctctgtgaccgccgcggacacggctgtatattactgtgcgagggactatggtccggggaattatgactggtacttcgatctctggggccgtggcaccctggtcactgtctcctcaggcggcggcggcagcggcggcggcggcagcggcggcggcggcagcgaaattgtgttgacacagtctccagccaccctgtctttgtctccaggggaaagagccaccctctcctgcagggccagtcagagtgttagcagctacttagcctggtaccaacagaaacctggccaggctcccaggctcctcatctatgatgcatccaacagggccactggcatcccagccaggttcagtggcagtgggtctgggacagacttcactctcaccatcagcagcctagagcctgaagattttgcagtttattactgtcagcagcgtagcaactggcctccggcgctcactttcggcggagggaccaaggtggagatcaaagccgaggccgccgccaaggaggccgccgccaaggccggacaaaacgacaccagccaaaccagcagcccctcagcatccagcaacataagcggaggcattttccttttcttcgtggccaatgccataatccacctcttctgcttcagttga

SEQ ID NO: 10 - protein, 318 aa, synthetic construct
  REGION 1..318: note = fusion protein
MKRFLFLLLTISLLVMVQIQTGLSQVQLQQWGAGLLKPSETLSLTCAVYGGSFSGYYWSWIRQSPEKGLEWIGEINHGGYVTYNPSLESRVTISVDTSKNQFSLKLSSVTAADTAVYYCARDYGPGNYDWYFDLWGRGTLVTVSSGGGGSGGGGSGGGGSEIVLTQSPATLSLSPGERATLSCRASQSVSSYLAWYQQKPGQAPRLLIYDASNRATGIPARFSGSGSGTDFTLTISSLEPEDFAVYYCQQRSNWPPALTFGGGTKVEIKAEAAAKEAAAKAGQNDTSQTSSPSASSNISGGIFLFFVANAIIHLFCFS

SEQ ID NO: 11 - DNA, 1836 bp, synthetic construct
  misc_feature 1..1836: note = TCR
  source 1..1836: mol_type = other DNA
atggagaccctcttgggcctgcttatcctttggctgcagctgcaatgggtgagcagcaaacaggaggtgacgcagattcctgcagctctgagtgtcccagaaggagaaaacttggttctcaactgcagtttcactgatagcgctatttacaacctccagtggtttaggcaggaccctgggaaaggtctcacatctctgttgcttattcagtcaagtcagagagagcaaacaagtggaagacttaatgcctcgctggataaatcatcaggacgtagtactttatacattgcagcttctcagcctggtgactcagccacctacctctgtgctgtgaggcccacatcaggaggaagctacatacctacatttggaagaggaaccagccttattgttcatccggatatccagaaccctgaccctgccgtgtaccagctgagagactctaaatccagtgacaagtctgtctgcctattcaccgattttgattctcaaacaaatgtgtcacaaagtaaggattctgatgtgtatatcacagacaaaactgtgctagacatgaggtctatggacttcaagagcaacagtgctgtggcctggagcaacaaatctgactttgcatgtgcaaacgccttcaacaacagcattattccagaagacaccttcttccccagcccagaaagttcctgtgatgtcaagctggtcgagaaaagctttgaaacagatacgaacctaaactttcaaaacctgtcagtgattgggttccgaatcctcctcctgaaagtggccgggtttaatctgctcatgacgctgcggctgtggtccagcgccaccaacttcagcctgctgaagcaggccggcgacgtggaggagaaccccggccccatgagcatcggcctcctgtgctgtgcagccttgtctctcctgtgggcaggtccagtgaatgctggtgtcactcagaccccaaaattccaggtcctgaagacaggacagagcatgacactgcagtgtgcccaggatatgaaccatgaatacatgtcctggtatcgacaagacccaggcatggggctgaggctgattcattactcagttggtgctggtatcactgaccaaggagaagtccccaatggctacaatgtctccagatcaaccacagaggatttcccgctcaggctgctgtcggctgctccctcccagacatctgtgtacttctgtgccagcagttacgtcgggaacaccggggagctgttttttggagaaggctctaggctgaccgtactggaggacctgaaaaacgtgttcccacccgaggtcgctgtgtttgagccatcagaagcagagatctcccacacccaaaaggccacactggtatgcctggccacaggcttctaccccgaccacgtggagctgagctggtgggtgaatgggaaggaggtgcacagtggggtcagcacagacccgcagcccctcaaggagcagcccgccctcaatgactccagatactgcctgagcagccgcctgagggtctcggccaccttctggcagaacccccgcaaccacttccgctgtcaagtccagttctacgggctctcggagaatgacgagtggacccaggatagggccaaacccgtcacccagatcgtcagcgccgaggcctggggtagagcagactgtggcttcacctccgagtcttaccagcaaggggtcctgtctgccaccatcctctatgagatcttgctagggaaggccaccttgtatgccgtgctggtcagtgccctcgtgctgatggctatggtcaagagaaaggattccagaggccgggccaagcggtccggatccgga

SEQ ID NO: 12 - DNA, 2610 bp, synthetic construct
  misc_feature 1..2610: note = TCR-EGFP
  source 1..2610: mol_type = other DNA
atggagaccctcttgggcctgcttatcctttggctgcagctgcaatgggtgagcagcaaacaggaggtgacgcagattcctgcagctctgagtgtcccagaaggagaaaacttggttctcaactgcagtttcactgatagcgctatttacaacctccagtggtttaggcaggaccctgggaaaggtctcacatctctgttgcttattcagtcaagtcagagagagcaaacaagtggaagacttaatgcctcgctggataaatcatcaggacgtagtactttatacattgcagcttctcagcctggtgactcagccacctacctctgtgctgtgaggcccacatcaggaggaagctacatacctacatttggaagaggaaccagccttattgttcatccggatatccagaaccctgaccctgccgtgtaccagctgagagactctaaatccagtgacaagtctgtctgcctattcaccgattttgattctcaaacaaatgtgtcacaaagtaaggattctgatgtgtatatcacagacaaaactgtgctagacatgaggtctatggacttcaagagcaacagtgctgtggcctggagcaacaaatctgactttgcatgtgcaaacgccttcaacaacagcattattccagaagacaccttcttccccagcccagaaagttcctgtgatgtcaagctggtcgagaaaagctttgaaacagatacgaacctaaactttcaaaacctgtcagtgattgggttccgaatcctcctcctgaaagtggccgggtttaatctgctcatgacgctgcggctgtggtccagcgccaccaacttcagcctgctgaagcaggccggcgacgtggaggagaaccccggccccatgagcatcggcctcctgtgctgtgcagccttgtctctcctgtgggcaggtccagtgaatgctggtgtcactcagaccccaaaattccaggtcctgaagacaggacagagcatgacactgcagtgtgcccaggatatgaaccatgaatacatgtcctggtatcgacaagacccaggcatggggctgaggctgattcattactcagttggtgctggtatcactgaccaaggagaagtccccaatggctacaatgtctccagatcaaccacagaggatttcccgctcaggctgctgtcggctgctccctcccagacatctgtgtacttctgtgccagcagttacgtcgggaacaccggggagctgttttttggagaaggctctaggctgaccgtactggaggacctgaaaaacgtgttcccacccgaggtcgctgtgtttgagccatcagaagcagagatctcccacacccaaaaggccacactggtatgcctggccacaggcttctaccccgaccacgtggagctgagctggtgggtgaatgggaaggaggtgcacagtggggtcagcacagacccgcagcccctcaaggagcagcccgccctcaatgactccagatactgcctgagcagccgcctgagggtctcggccaccttctggcagaacccccgcaaccacttccgctgtcaagtccagttctacgggctctcggagaatgacgagtggacccaggatagggccaaacccgtcacccagatcgtcagcgccgaggcctggggtagagcagactgtggcttcacctccgagtcttaccagcaaggggtcctgtctgccaccatcctctatgagatcttgctagggaaggccaccttgtatgccgtgctggtcagtgccctcgtgctgatggctatggtcaagagaaaggattccagaggccgggccaagcggtccggatccggagccaccaacttcagcctgctgaagcaggccggcgacgtggaggagaaccccggccccatgtccaagggcgaggaactgttcacgggcgtcgtcccgatcctcgtcgaactcgatggcgacgtcaacggccacaagttctccgtcagcggtgaaggtgaaggcgacgccacctacggcaagctcacccttaagttcatctgcaccaccggcaaactgccggtgccgtggccgacgctggtcacgaccctcacgtatggcgttcagtgcttctcgcgctacccggaccacatgaagcagcacgatttcttcaagtcggcgatgccggaaggctacgtccaggaacgcacgatcttcttcaaggacgatggcaactacaagacccgcgccgaagtcaagttcgagggcgacacgcttgtgaatcgcatcgaacttaagggcatcgacttcaaggaagatggcaacatcctcggccacaagctggagtataactacaattcgcacaacgtctacatcatggctgacaagcagaagaatggtatcaaggttaacttcaagatccgccacaacatcgaagacggctccgtccagctggcggaccactatcagcagaacaccccgatcggcgacggcccggttctcctcccggataaccactacctcagcacgcagtcggcgctgtcgaaggacccgaatgaaaagcgcgaccacatggtccttctggagttcgtgaccgcggcgggcatcacgcacggcatggacgaactttacaagtaa

SEQ ID NO: 13 - DNA, 808 bp, synthetic construct
  misc_feature 1..808: note = encoding nucleic acids
  source 1..808: mol_type = other DNA
atgtgctccagaggttgggattcgtgtctggctctggaattgctactgctgcctctgtcactcctggtgaccagcattcgattgtgatattgaaggtaaagatggcaaacaatatgagagtgttctaatggtcagcatcgatcaattattggacagcatgaaagaaattggtagcaattgcctgaataatgaatttaacttttttaaaagacatatctgtgatgctaataaggaaggtatgtttttattccgtgctgctcgcaagttgaggcaatttcttaaaatgaatagcactggtgattttgatctccacttattaaaagtttcagaaggcacaacaatactgttgaactgcactggccaggttaaaggaagaaaaccagctgccctgggtgaagcccaaccaacaaagagtttggaagaaaataaatctttaaaggaacagaaaaaactgaatgacttgtgtttcctaaagagactattacaagagataaaaacttgttggaataaaattttgatgggcactaaagaacacttcgtgccggtcttcctgccagcgaagcccaccacgacgccagcgccgcgaccaccaacaccggcgcccaccatcgcgtcgcagcccctgtccctgcgcccagaggcgtgccggccagcggcggggggcgcagtgcacacgagggggctggacttcgcctgtgatgatgtgtgcagtccaccctgtaccctggcccggtcctttggagtagaatggattgcaagttggctagtggtcacggtgcccaccattcttggcctgttacttacctaa

SEQ ID NO: 14 - protein, 268 aa, synthetic construct
  REGION 1..268: note = fusion protein
MCSRGWDSCLALELLLLPLSLLVTSIDCDIEGKDGKQYESVLMVSIDQLLDSMKEIGSNCLNNEFNFFKRHICDANKEGMFLFRAARKLRQFLKMNSTGDFDLHLLKVSEGTTILLNCTGQVKGRKPAALGEAQPTKSLEENKSLKEQKKLNDLCFLKRLLQEIKTCWNKILMGTKEHFVPVFLPAKPTTTPAPRPPTPAPTIASQPLSLRPEACRPAAGGAVHTRGLDFACDDVCSPPCTLARSFGVEWIASWLVVTVPTILGLLLT

SEQ ID NO: 15 - DNA, 849 bp, synthetic construct
  misc_feature 1..849: note = encoding nucleic acids
  source 1..849: mol_type = other DNA
atgaccgtcgcgcggccgagcgtgcccgcggcgctgcccctcctcggggagctgccccggctgctgctgctggtgctgttgtgcctgccggccgtgtggggtgattgtgatattgaaggtaaagatggcaaacaatatgagagtgttctaatggtcagcatcgatcaattattggacagcatgaaagaaattggtagcaattgcctgaataatgaatttaacttttttaaaagacatatctgtgatgctaataaggaaggtatgtttttattccgtgctgctcgcaagttgaggcaatttcttaaaatgaatagcactggtgattttgatctccacttattaaaagtttcagaaggcacaacaatactgttgaactgcactggccaggttaaaggaagaaaaccagctgccctgggtgaagcccaaccaacaaagagtttggaagaaaataaatctttaaaggaacagaaaaaactgaatgacttgtgtttcctaaagagactattacaagagataaaaacttgttggaataaaattttgatgggcactaaagaacacttcgtgccggtcttcctgccagcgaagcccaccacgacgccagcgccgcgaccaccaacaccggcgcccaccatcgcgtcgcagcccctgtccctgcgcccagaggcgtgccggccagcggcggggggcgcagtgcacacgagggggctggacttcgcctgtgatcatgaaacaaccccaaataaaggaagtggaaccacttcaggtactacccgtcttctatctgggcacacgtgtttcacgttgacaggtttgcttgggacgctagtaaccatgggcttgctgacttaa

SEQ ID NO: 16 - protein, 282 aa, synthetic construct
  REGION 1..282: note = fusion protein
MTVARPSVPAALPLLGELPRLLLLVLLCLPAVWGDCDIEGKDGKQYESVLMVSIDQLLDSMKEIGSNCLNNEFNFFKRHICDANKEGMFLFRAARKLRQFLKMNSTGDFDLHLLKVSEGTTILLNCTGQVKGRKPAALGEAQPTKSLEENKSLKEQKKLNDLCFLKRLLQEIKTCWNKILMGTKEHFVPVFLPAKPTTTPAPRPPTPAPTIASQPLSLRPEACRPAAGGAVHTRGLDFACDHETTPNKGSGTTSGTTRLLSGHTCFTLTGLLGTLVTMGLLT

SEQ ID NO: 17 - DNA, 813 bp, synthetic construct
  misc_feature 1..813: note = encoding nucleic acids
  source 1..813: mol_type = other DNA
atgctggggccctgcatgctgctgctgctgctgctgggcctgaggctacagctctccctgggcgattgtgatattgaaggtaaagatggcaaacaatatgagagtgttctaatggtcagcatcgatcaattattggacagcatgaaagaaattggtagcaattgcctgaataatgaatttaacttttttaaaagacatatctgtgatgctaataaggaaggtatgtttttattccgtgctgctcgcaagttgaggcaatttcttaaaatgaatagcactggtgattttgatctccacttattaaaagtttcagaaggcacaacaatactgttgaactgcactggccaggttaaaggaagaaaaccagctgccctgggtgaagcccaaccaacaaagagtttggaagaaaataaatctttaaaggaacagaaaaaactgaatgacttgtgtttcctaaagagactattacaagagataaaaacttgttggaataaaattttgatgggcactaaagaacacttcgtgccggtcttcctgccagcgaagcccaccacgacgccagcgccgcgaccaccaacaccggcgcccaccatcgcgtcgcagcccctgtccctgcgcccagaggcgtgccggccagcggcggggggcgcagtgcacacgagggggctggacttcgcctgtgataccgcctgcgacctggcgccccccgccggcaccaccgacgccgcgcacccggggccgtccgtggtccccgcgttgcttcctctgctggcagggaccttgctgctgctggggacggccactgctccctaa

SEQ ID NO: 18 - protein, 270 aa, synthetic construct
  REGION 1..270: note = fusion protein
MLGPCMLLLLLLGLRLQLSLGDCDIEGKDGKQYESVLMVSIDQLLDSMKEIGSNCLNNEFNFFKRHICDANKEGMFLFRAARKLRQFLKMNSTGDFDLHLLKVSEGTTILLNCTGQVKGRKPAALGEAQPTKSLEENKSLKEQKKLNDLCFLKRLLQEIKTCWNKILMGTKEHFVPVFLPAKPTTTPAPRPPTPAPTIASQPLSLRPEACRPAAGGAVHTRGLDFACDTACDLAPPAGTTDAAHPGPSVVPALLPLLAGTLLLLGTATAP

SEQ ID NO: 19 - DNA, 810 bp, synthetic construct
  misc_feature 1..810: note = encoding nucleic acids
  source 1..810: mol_type = other DNA
atgaacctggccatcagcatcgctctcctgctaacagtcttgcaggtctcccgaggggattgtgatattgaaggtaaagatggcaaacaatatgagagtgttctaatggtcagcatcgatcaattattggacagcatgaaagaaattggtagcaattgcctgaataatgaatttaacttttttaaaagacatatctgtgatgctaataaggaaggtatgtttttattccgtgctgctcgcaagttgaggcaatttcttaaaatgaatagcactggtgattttgatctccacttattaaaagtttcagaaggcacaacaatactgttgaactgcactggccaggttaaaggaagaaaaccagctgccctgggtgaagcccaaccaacaaagagtttggaagaaaataaatctttaaaggaacagaaaaaactgaatgacttgtgtttcctaaagagactattacaagagataaaaacttgttggaataaaattttgatgggcactaaagaacacttcgtgccggtcttcctgccagcgaagcccaccacgacgccagcgccgcgaccaccaacaccggcgcccaccatcgcgtcgcagcccctgtccctgcgcccagaggcgtgccggccagcggcggggggcgcagtgcacacgagggggctggacttcgcctgtgataacgtcacagtgctcagagacaaactggtcaagtgtgagggcatcagcctgctggctcagaacacctcgtggctgctgctgctcctgctctccctctccctcctccaggccacggatttcatgtccctgtaa

SEQ ID NO: 20 - protein, 269 aa, synthetic construct
  REGION 1..269: note = fusion protein
MNLAISIALLLTVLQVSRGDCDIEGKDGKQYESVLMVSIDQLLDSMKEIGSNCLNNEFNFFKRHICDANKEGMFLFRAARKLRQFLKMNSTGDFDLHLLKVSEGTTILLNCTGQVKGRKPAALGEAQPTKSLEENKSLKEQKKLNDLCFLKRLLQEIKTCWNKILMGTKEHFVPVFLPAKPTTTPAPRPPTPAPTIASQPLSLRPEACRPAAGGAVHTRGLDFACDNVTVLRDKLVKCEGISLLAQNTSWLLLLLLSLSLLQATDFMSL